European Patent Specification EP 3 630 175 B1, published March 11, 2026. Title: METHODS AND DEVICES FOR THE TREATMENT OF FOOD ALLERGIES. Applicant: GILL, HARVINDER SINGH SHAKYA, AKHILESH. Application UNKNOWN. The sequence listing filed with the application follows.

SEQUENCE LISTING (28 sequences)

SEQ ID NO: 1 - protein, 8 aa, Artificial Sequence
  Synthetic peptide
PGQFEDFF

SEQ ID NO: 2 - protein, 8 aa, Artificial Sequence
  Synthetic peptide
YLQGFSRN

SEQ ID NO: 3 - protein, 10 aa, Artificial Sequence
  Synthetic peptide
FNAEFNEIRR

SEQ ID NO: 4 - protein, 8 aa, Artificial Sequence
  Synthetic peptide
QEERGQRR

SEQ ID NO: 5 - protein, 10 aa, Artificial Sequence
  Synthetic peptide
DITNPINLRE

SEQ ID NO: 6 - protein, 10 aa, Artificial Sequence
  Synthetic peptide
NNFGKLFEVK

SEQ ID NO: 7 - protein, 6 aa, Artificial Sequence
  Synthetic peptide
GNLELV

SEQ ID NO: 8 - protein, 10 aa, Artificial Sequence
  Synthetic peptide
RRYTARLKEG

SEQ ID NO: 9 - protein, 10 aa, Artificial Sequence
  Synthetic peptide
ELHLLGFGIN

SEQ ID NO: 10 - protein, 10 aa, Artificial Sequence
  Synthetic peptide
HRIFLAGDKD

SEQ ID NO: 11 - protein, 10 aa, Artificial Sequence
  Synthetic peptide
IDQIEKQAKD

SEQ ID NO: 12 - protein, 10 aa, Artificial Sequence
  Synthetic peptide
KDLAFPGSGE

SEQ ID NO: 13 - protein, 10 aa, Artificial Sequence
  Synthetic peptide
KESHFVSARP

SEQ ID NO: 14 - protein, 25 aa, Artificial Sequence
  Synthetic peptide
NEGVIVKVSKEHVEELTKHAKSVSK

SEQ ID NO: 15 - protein, 10 aa, Artificial Sequence
  Synthetic peptide
HASARQQWEL

SEQ ID NO: 16 - protein, 10 aa, Artificial Sequence
  Synthetic peptide
QWELQGDRRC

SEQ ID NO: 17 - protein, 10 aa, Artificial Sequence
  Synthetic peptide
DRRCQSQLER

SEQ ID NO: 18 - protein, 10 aa, Artificial Sequence
  Synthetic peptide
LRPCEQHLMQ

SEQ ID NO: 19 - protein, 10 aa, Artificial Sequence
  Synthetic peptide
KIQRDEDSYE

SEQ ID NO: 20 - protein, 10 aa, Artificial Sequence
  Synthetic peptide
YERDPYSPSQ

SEQ ID NO: 21 - protein, 10 aa, Artificial Sequence
  Synthetic peptide
SQDPYSPSPY

SEQ ID NO: 22 - protein, 10 aa, Artificial Sequence
  Synthetic peptide
DRLQGRQQEQ

SEQ ID NO: 23 - protein, 10 aa, Artificial Sequence
  Synthetic peptide
KRELRNLPQQ

SEQ ID NO: 24 - protein, 10 aa, Artificial Sequence
  Synthetic peptide
QRCDLDVESG

SEQ ID NO: 25 - protein, 15 aa, Artificial Sequence
  Synthetic peptide
IETWNPNNQEFECAG

SEQ ID NO: 26 - protein, 15 aa, Artificial Sequence
  Synthetic peptide
GNIFSGFTPEFLAQA

SEQ ID NO: 27 - protein, 15 aa, Artificial Sequence
  Synthetic peptide
VTVRGGLRILSPDRK

SEQ ID NO: 28 - protein, 15 aa, Artificial Sequence
  Synthetic peptide
DEDEYEYDEEDRRRG